European Patent Specification EP 3 191 484 B1, published June 12, 2024. Title: Pyrazolopyridine derivatives and their use in therapy. Applicant: Helmholtz Zentrum München - Deutsches Forschungszentrum für Gesundheit und Umwelt (GmbH), et al. The sequence listing filed with the application follows.

SEQUENCE LISTING (5 sequences)

SEQ ID NO: 1 - protein, 51 aa, Trypanosoma brucei
EKRVSNAVEFLLDSRVRRTPTSSKVHFLKSKGLSAEEICEAFTKVGQPKTL

SEQ ID NO: 2 - protein, 48 aa, Trypanosoma cruzi
RKRVSSAVQFLHDSRVKITPAANKIQFLKSKGLTTEEVCEAFEKAGQT

SEQ ID NO: 3 - protein, 46 aa, Trypanosoma congolense
KAQRIANAVEFLLDPRVKNASTANKVRFLKSKNLSAEEICEAFVKC

SEQ ID NO: 4 - protein, 50 aa, Leishmania donovani
DADPTVQSAIRFLQDSRVRRSPVESQIRFLKGKGVPDEQIKYALAKVGRA

SEQ ID NO: 5 - protein, 48 aa, Homo sapiens
EPLIATAVKFLQNSRVRQSPLATRRAFLKKKGLTDEEIDMAFQQSGTA